European Patent Application EP 4 772 538 A1, published July 8, 2026. Title: 结合HLA-A02/MAGE-A4复合体的多种抗体及其用途. Applicant: 北京智仁美博生物科技有限公司. The sequence listing filed with the application follows.

SEQUENCE LISTING (94 sequences)

SEQ ID NO: 1 - protein, 10 aa, homo sapiens
GVYDGREHTV

SEQ ID NO: 2 - protein, 10 aa, homo sapiens
GLYDGREHSV

SEQ ID NO: 3 - protein, 10 aa, homo sapiens
EVYDGREHSA

SEQ ID NO: 4 - protein, 10 aa, homo sapiens
ISYSGVLHAV

SEQ ID NO: 5 - protein, 10 aa, homo sapiens
GGYPGGIHEV

SEQ ID NO: 6 - protein, 11 aa, homo sapiens
YLISQVEGHQV

SEQ ID NO: 7 - protein, 10 aa, homo sapiens
DSYGGRHHRL

SEQ ID NO: 8 - protein, 10 aa, homo sapiens
VGYPGRLHLW

SEQ ID NO: 9 - protein, 10 aa, homo sapiens
FVYDEPGHAV

SEQ ID NO: 10 - protein, 10 aa, homo sapiens
SQYSGQLHEV

SEQ ID NO: 11 - protein, 9 aa, homo sapiens
ALYGRLEVV

SEQ ID NO: 12 - protein, 10 aa, homo sapiens
NTYEGRPIYV

SEQ ID NO: 13 - protein, 10 aa, homo sapiens
NTYEGRPIYV

SEQ ID NO: 14 - protein, 9 aa, homo sapiens
KIYEGAYHV

SEQ ID NO: 15 - protein, 9 aa, homo sapiens
RLYTGMHTV

SEQ ID NO: 16 - protein, 10 aa, homo sapiens
GVYAGRPLSV

SEQ ID NO: 17 - protein, 10 aa, homo sapiens
GVYQGRVSAV

SEQ ID NO: 18 - protein, 10 aa, homo sapiens
AVLDGRELRV

SEQ ID NO: 19 - protein, 9 aa, homo sapiens
RLYDGLFKV

SEQ ID NO: 20 - protein, 9 aa, homo sapiens
DVYDGRFLV

SEQ ID NO: 21 - protein, 9 aa, homo sapiens
SRYDGQIAV

SEQ ID NO: 22 - protein, 9 aa, homo sapiens
NRYDGIYKV

SEQ ID NO: 23 - protein, 9 aa, homo sapiens
NRYDGQVAV

SEQ ID NO: 24 - protein, 9 aa, homo sapiens
LMYDGTKEV

SEQ ID NO: 25 - protein, 11 aa, homo sapiens
HVYDGKFLARV

SEQ ID NO: 26 - protein, 10 aa, homo sapiens
YIYDGELVSK

SEQ ID NO: 27 - protein, 10 aa, homo sapiens
ATYDGQFMKL

SEQ ID NO: 28 - protein, 9 aa, homo sapiens
FAYDGKDYL

SEQ ID NO: 29 - protein, 9 aa, homo sapiens
KLYDGFQYL

SEQ ID NO: 30 - protein, 9 aa, homo sapiens
SVYDGKLLI

SEQ ID NO: 31 - protein, 9 aa, homo sapiens
YAYDGKDYI

SEQ ID NO: 32 - protein, 5 aa, Camelus
DSDMG

SEQ ID NO: 33 - protein, 16 aa, Camelus
TITTDGSTYYADSVKG

SEQ ID NO: 34 - protein, 18 aa, Camelus
DLPILRPTPCGDSVLYNY

SEQ ID NO: 35 - protein, 126 aa, Camelus
EVQLVESGGGSVQTGETLRLSCTVSGFTFDDSDMGWYRQAPGNECELVSTITTDGSTYYADSVKGRFTISQDNAKTTAYLQMDSLKPEDTAVYYCAADLPILRPTPCGDSVLYNYWGQGTQVTVSS

SEQ ID NO: 36 - protein, 126 aa, synthetic construct
QVQLVESGGGLVKPGGSLRLSCAVSGFTFDDSDMGWYRQAPGNECELVSTITTDGSTYYADSVKGRFTISQDNAKTSAYLQMNSLRAEDTAVYYCAADLPILRPTPCGDSVLYNYWGQGTTVTVSS

SEQ ID NO: 37 - protein, 5 aa, synthetic construct
GYTMN

SEQ ID NO: 38 - protein, 17 aa, synthetic construct
LINPYKGVSTYNQKFKD

SEQ ID NO: 39 - protein, 13 aa, synthetic construct
SGYYGDSDWYFDV

SEQ ID NO: 40 - protein, 11 aa, synthetic construct
RASQDIRNYLN

SEQ ID NO: 41 - protein, 7 aa, synthetic construct
YTSRLES

SEQ ID NO: 42 - protein, 9 aa, synthetic construct
QQGNTLPWT

SEQ ID NO: 43 - protein, 122 aa, synthetic construct [sequence omitted]

SEQ ID NO: 44 - protein, 107 aa, synthetic construct [sequence omitted]

SEQ ID NO: 45 - protein, 498 aa, synthetic construct
QVQLVESGGGLVKPGGSLRLSCAVSGFTFDDSDMGWYRQAPGNECELVSTITTDGSTYYADSVKGRFTISQDNAKTSAYLQMNSLRAEDTAVYYCAADLPILRPTPCGDSVLYNYWGQGTTVTVSSGGGGSGGGGSGGGGSQVQLVESGGGLVKPGGSLRLSCAVSGFTFDDSDMGWYRQAPGNECELVSTITTDGSTYYADSVKGRFTISQDNAKTSAYLQMNSLRAEDTAVYYCAADLPILRPTPCGDSVLYNYWGQGTTVTVSSASERKSSVECPPCPAPEFEGGPSVFLFPPKPKDTLMISRTPEVTCVVVDVSQEDPEVQFNWYVDGVEVHNAKTKPREEQYNSTYRVVSVLTVLHQDWLNGKEYKCKVSNKALPASIEKTISKAKGQPREPQVCTLPPSQEEMTKNQVSLSCAVKGFYPSDIAVEWESNGQPENNYKTTPPVLDSDGSFFLVSKLTVDKSRWQEGNVFSCSVMHEALHNHYTQKSLSLSPGK

SEQ ID NO: 46 - protein, 484 aa, synthetic construct
DIQMTQSPSSLSASVGDRVTITCRASQDIRNYLNWYQQKPGKAPKLLIYYTSRLESGVPSRFSGSGSGTDYTLTISSLQPEDFATYYCQQGNTLPWTFGQGTKVEIKGGGGSGGGGSGGGGSGGGGSGGGSEVQLVESGGGLVQPGGSLRLSCAASGYSFTGYTMNWVRQAPGKGLEWVALINPYKGVSTYNQKFKDRFTISVDKSKNTAYLQMNSLRAEDTAVYYCARSGYYGDSDWYFDVWGQGTLVTVSSASERKSSVECPPCPAPEFEGGPSVFLFPPKPKDTLMISRTPEVTCVVVDVSHEDPEVKFNWYVDGVEVHNAKTKPREEQYNSTYRVVSVLTVLHQDWLNGKEYKCKVSNKALPASIEKTISKAKGQPREPQVYTLPPCREEMTKNQVSLWCLVKGFYPSDIAVEWESNGQPENNYKTTPPVLDSDGSFFLYSKLTVDKSRWQQGNVFSCSVMHEALHNHYTQKSLSLSPGK

SEQ ID NO: 47 - protein, 419 aa, synthetic construct
GVYDGREHTVGCGGSGGGGSGGGGSIQRTPKIQVYSRHPAENGKSNFLNCYVSGFHPSDIEVDLLKNGERIEKVEHSDLSFSKDWSFYLLYYTEFTPTEKDEYACRVNHVTLSQPKIVKWDRDMGGGGSGGGGSGGGGSGGGGSGSHSMRYFFTSVSRPGRGEPRFIAVGYVDDTQFVRFDSDAASQRMEPRAPWIEQEGPEYWDGETRKVKAHSQTHRVDLGTLRGCYNQSEAGSHTVQRMYGCDVGSDWRFLRGYHQYAYDGKDYIALKEDLRSWTAADMAAQTTKHKWEAAHVAEQLRAYLEGTCVEWLRRYLENGKETLQRTDAPKTHMTHHAVSDHEATLRCWALSFYPAEITLTWQRDGEDQTQDTELVETRPAGDGTFQKWAAVVVPSGQEQRYTCHVQHEGLPKPLTLRWE

SEQ ID NO: 48 - protein, 317 aa, homo sapiens
MSSEQKSQHCKPEEGVEAQEEALGLVGAQAPTTEEQEAAVSSSSPLVPGTLEEVPAAESAGPPQSPQGASALPTTISFTCWRQPNEGSSSQEEEGPSTSPDAESLFREALSNKVDELAHFLLRKYRAKELVTKAEMLERVIKNYKRCFPVIFGKASESLKMIFGIDVKEVDPASNTYTLVTCLGLSYDGLLGNNQIFPKTGLLIIVLGTIAMEGDSASEEEIWEELGVMGVYDGREHTVYGEPRKLLTQDWVQENYLEYRQVPGSNPARYEFLWGPRALAETSYVKVLEHVVRVNARVRIAYPSLREAALLEEEEGV

SEQ ID NO: 49 - protein, 15 aa, synthetic construct
GGGGSGGGGSGGGGS

SEQ ID NO: 50 - DNA, 22 bp, synthetic construct
  source 1..22: mol_type = other DNA
tccttccccgtcagccagtcct

SEQ ID NO: 51 - protein, 105 aa, homo sapiens
QDGNEEMGGITQTPYKVSISGTTVILTCPQYPGSEILWQHNDKNIGGDEDDKNIGSDEDHLSLKEFSELEQSGYYVCYPRGSKPEDANFYLYLRARVCENCMEMD

SEQ ID NO: 52 - protein, 84 aa, homo sapiens [sequence omitted]

SEQ ID NO: 53 - protein, 6 aa, synthetic construct
HHHHHH

SEQ ID NO: 54 - protein, 234 aa, homo sapiens
ASEPKSSDKTHTCPPCPAPELLGGPSVFLFPPKPKDTLMISRTPEVTCVVVDVSHEDPEVKFNWYVDGVEVHNAKTKPREEQYNSTYRVVSVLTVLHQDWLNGKEYKCKVSNKALPAPIEKTISKAKGQPREPQVYTLPPSRDELTKNQVSLTCLVKGFYPSDIAVEWESNGQPENNYKTTPPVLDSDGSFFLYSKLTVDKSRWQQGNVFSCSVMHEALHNHYTQKSLSLSPGK

SEQ ID NO: 55 - protein, 234 aa, mus musculus
ASPRGPTIKPCPPCKCPAPNLLGGPSVFIFPPKIKDVLMISLSPIVTCVVVDVSEDDPDVQISWFVNNVEVHTAQTQTHREDYNSTLRVVSALPIQHQDWMSGKEFKCKVNNKDLPAPIERTISKPKGSVRAPQVYVLPPPEEEMTKKQVTLTCMVTDFMPEDIYVEWTNNGKTELNYKNTEPVLDSDGSYFMYSKLRVEKKNWVERNSYSCSVVHEGLHNHHTTKSFSRTPGK

SEQ ID NO: 56 - protein, 330 aa, homo sapiens
ASTKGPSVFPLAPSSKSTSGGTAALGCLVKDYFPEPVTVSWNSGALTSGVHTFPAVLQSSGLYSLSSVVTVPSSSLGTQTYICNVNHKPSNTKVDKRVEPKSCDKTHTCPPCPAPELLGGPSVFLFPPKPKDTLMISRTPEVTCVVVDVSHEDPEVKFNWYVDGVEVHNAKTKPREEQYNSTYRVVSVLTVLHQDWLNGKEYKCKVSNKALPAPIEKTISKAKGQPREPQVYTLPPSREEMTKNQVSLTCLVKGFYPSDIAVEWESNGQPENNYKTTPPVLDSDGSFFLYSKLTVDKSRWQQGNVFSCSVMHEALHNHYTQKSLSLSPGK

SEQ ID NO: 57 - protein, 330 aa, synthetic construct
ASTKGPSVFPLAPSSKSTSGGTAALGCLVKDYFPEPVTVSWNSGALTSGVHTFPAVLQSSGLYSLSSVVTVPSSSLGTQTYICNVNHKPSNTKVDKRVEPKSCDKTHTCPPCPAPELLGGPSVFLFPPKPKDTLMISRTPEVTCVVVDVSHEDPEVKFNWYVDGVEVHNAKTKPREEQYNSTYRVVSVLTVLHQDWLNGKEYKCKVSNKALPAPIEKTISKAKGQPREPQVCTLPPSREEMTKNQVSLSCAVKGFYPSDIAVEWESNGQPENNYKTTPPVLDSDGSFFLVSKLTVDKSRWQQGNVFSCSVMHEALHNHYTQKSLSLSPGK

SEQ ID NO: 58 - protein, 330 aa, synthetic construct
ASTKGPSVFPLAPSSKSTSGGTAALGCLVKDYFPEPVTVSWNSGALTSGVHTFPAVLQSSGLYSLSSVVTVPSSSLGTQTYICNVNHKPSNTKVDKRVEPKSCDKTHTCPPCPAPELLGGPSVFLFPPKPKDTLMISRTPEVTCVVVDVSHEDPEVKFNWYVDGVEVHNAKTKPREEQYNSTYRVVSVLTVLHQDWLNGKEYKCKVSNKALPAPIEKTISKAKGQPREPQVYTLPPCREEMTKNQVSLWCLVKGFYPSDIAVEWESNGQPENNYKTTPPVLDSDGSFFLYSKLTVDKSRWQQGNVFSCSVMHEALHNHYTQKSLSLSPGK

SEQ ID NO: 59 - protein, 330 aa, synthetic construct
ASTKGPSVFPLAPSSKSTSGGTAALGCLVKDYFPEPVTVSWNSGALTSGVHTFPAVLQSSGLYSLSSVVTVPSSSLGTQTYICNVNHKPSNTKVDKRVEPKSCDKTHTCPPCPAPEFEGGPSVFLFPPKPKDTLMISRTPEVTCVVVDVSHEDPEVKFNWYVDGVEVHNAKTKPREEQYNSTYRVVSVLTVLHQDWLNGKEYKCKVSNKALPASIEKTISKAKGQPREPQVCTLPPSREEMTKNQVSLSCAVKGFYPSDIAVEWESNGQPENNYKTTPPVLDSDGSFFLVSKLTVDKSRWQQGNVFSCSVMHEALHNHYTQKSLSLSPGK

SEQ ID NO: 60 - protein, 330 aa, synthetic construct
ASTKGPSVFPLAPSSKSTSGGTAALGCLVKDYFPEPVTVSWNSGALTSGVHTFPAVLQSSGLYSLSSVVTVPSSSLGTQTYICNVNHKPSNTKVDKRVEPKSCDKTHTCPPCPAPEFEGGPSVFLFPPKPKDTLMISRTPEVTCVVVDVSHEDPEVKFNWYVDGVEVHNAKTKPREEQYNSTYRVVSVLTVLHQDWLNGKEYKCKVSNKALPASIEKTISKAKGQPREPQVYTLPPCREEMTKNQVSLWCLVKGFYPSDIAVEWESNGQPENNYKTTPPVLDSDGSFFLYSKLTVDKSRWQQGNVFSCSVMHEALHNHYTQKSLSLSPGK

SEQ ID NO: 61 - protein, 327 aa, synthetic construct
ASTKGPSVFPLAPSSKSTSEGTAALGCLVKDYFPEPVTVSWNSGALTSGVHTFPAVLQSSGLYSLSSVVTVPSSSLGTQTYICNVDHKPSNTKVDKTVERKSCVECPPCPAPEFEGGPSVFLFPPKPKDTLMISRTPEVTCVVVDVSQEDPEVQFNWYVDGVEVHNAKTKPREEQYNSTYRVVSVLTVLHQDWLNGKEYKCKVSNKALPASIEKTISKAKGQPREPQVCTLPPSQEEMTKNQVSLSCAVKGFYPSDIAVEWESNGQPENNYKTTPPVLDSDGSFFLVSKLTVDKSRWQEGNVFSCSVMHEALHNHYTQKSLSLSPGK

SEQ ID NO: 62 - protein, 327 aa, synthetic construct
ASTKGPSVFPLAPSSKSTSGGTAALGCLVKDYFPEPVTVSWNSGALTSGVHTFPAVLQSSGLYSLSSVVTVPSSSLGTQTYICNVNHKPSNTKVDKRVERKSCVECPPCPAPEFEGGPSVFLFPPKPKDTLMISRTPEVTCVVVDVSHEDPEVKFNWYVDGVEVHNAKTKPREEQYNSTYRVVSVLTVLHQDWLNGKEYKCKVSNKALPASIEKTISKAKGQPREPQVYTLPPCREEMTKNQVSLWCLVKGFYPSDIAVEWESNGQPENNYKTTPPVLDSDGSFFLYSKLTVDKSRWQQGNVFSCSVMHEALHNHYTQKSLSLSPGK

SEQ ID NO: 63 - protein, 108 aa, homo sapiens
VLGQPKAAPSVTLFPPSSEELQANKATLVCLISDFYPGAVTVAWKADSSPVKAGVETTTPSKQSNNKYAASSYLSLTPEQWKSHRSYSCQVTHEGSTVEKTVAPTECS

SEQ ID NO: 64 - protein, 105 aa, homo sapiens [sequence omitted]

SEQ ID NO: 65 - protein, 115 aa, synthetic construct
EVQLLESGGGLVQPGGSLRLSCAASGFTFSSYAMSWVRQAPGKGLEWVSAISGSGGSTYYADSVKGRFTISRDNSKNTLYLQMNSLRAEDTAVYYCAKGSGFDYWGQGTLVTVSS

SEQ ID NO: 66 - protein, 108 aa, synthetic construct
EIVLTQSPGTLSLSPGERATLSCRASQSVSSSYLAWYQQKPGQAPRLLIYGASSRATGIPDRFSGSGSGTDFTLTISRLEPEDFAVYYCQQYGSSPLTFGQGTKVEIK

SEQ ID NO: 67 - protein, 113 aa, synthetic construct
ANQVEQSPQSLIILEGKNVTLQCNYTVSPFSNLRWYKQDTGRGPVSLTILDYAINTKSNGRYTATLDADTKQSSLHITASQLSDSASYICVVNRADGLYIPTFGRGTSLIVHP

SEQ ID NO: 68 - protein, 116 aa, synthetic construct
DVKVTQSSRYLVKRTGEKVFLECVQDAPLSKMFWYRQDPGLGLRLIYFSYDVKMKEKGDIPEGYSVSREKKERFSLILESASTNQTSMYLCASSSDQNSGDPYEQYFGPGTRLTVT

SEQ ID NO: 69 - protein, 444 aa, synthetic construct
ANQVEQSPQSLIILEGKNVTLQCNYTVSPFSNLRWYKQDTGRGPVSLTILDYAINTKSNGRYTATLDADTKQSSLHITASQLSDSASYICVVNRADGLYIPTFGRGTSLIVHPYIQNPDPAVYQLRDSKSSDKFVCLFTDFDSQINVSQSKDSDVYITDKCVLDMRSMDFKSNSAVAWSNKSDFTCANAFNNSIIPEDTFFPSPESSCGGGGSASERKSSVECPPCPAPEFEGGPSVFLFPPKPKDTLMISRTPEVTCVVVDVSHEDPEVKFNWYVDGVEVHNAKTKPREEQYNSTYRVVSVLTVLHQDWLNGKEYKCKVSNKALPASIEKTISKAKGQPREPQVYTLPPCREEMTKNQVSLWCLVKGFYPSDIAVEWESNGQPENNYKTTPPVLDSDGSFFLYSKLTVDKSRWQQGNVFSCSVMHEALHNHYTQKSLSLSPGK

SEQ ID NO: 70 - protein, 483 aa, synthetic construct
DVKVTQSSRYLVKRTGEKVFLECVQDAPLSKMFWYRQDPGLGLRLIYFSYDVKMKEKGDIPEGYSVSREKKERFSLILESASTNQTSMYLCASSSDQNSGDPYEQYFGPGTRLTVTEDLKNVFPPEVAVFEPSKAEISRTQKATLVCLATGFYPPHVELSWWVNGKEVHDGVCTDPQPLKEQPALNDSRYALSSRLRVSATFWQDPRNHFRCQVQFYGLSENDEWTQDRAKPVTQIVSAEAWGRADCGGGGSASERKSCVECPPCPAPEFEGGPSVFLFPPKPKDTLMISRTPEVTCVVVDVSQEDPEVQFNWYVDGVEVHNAKTKPREEQYNSTYRVVSVLTVLHQDWLNGKEYKCKVSNKALPASIEKTISKAKGQPREPQVCTLPPSQEEMTKNQVSLSCAVKGFYPSDIAVEWESNGQPENNYKTTPPVLDSDGSFFLVSKLTVDKSRWQEGNVFSCSVMHEALHNHYTQKSLSLSPGK

SEQ ID NO: 71 - protein, 267 aa, synthetic construct
EVQLVESGGGSVQTGETLRLSCTVSGFTFDDSDMGWYRQAPGNECELVSTITTDGSTYYADSVKGRFTISQDNAKTTAYLQMDSLKPEDTAVYYCAADLPILRPTPCGDSVLYNYWGQGTQVTVSSGGGGSGGGGSGGGGSEVQLVESGGGSVQTGETLRLSCTVSGFTFDDSDMGWYRQAPGNECELVSTITTDGSTYYADSVKGRFTISQDNAKTTAYLQMDSLKPEDTAVYYCAADLPILRPTPCGDSVLYNYWGQGTQVTVSS

SEQ ID NO: 72 - protein, 267 aa, synthetic construct
QVQLVESGGGLVKPGGSLRLSCAVSGFTFDDSDMGWYRQAPGNECELVSTITTDGSTYYADSVKGRFTISQDNAKTSAYLQMNSLRAEDTAVYYCAADLPILRPTPCGDSVLYNYWGQGTTVTVSSGGGGSGGGGSGGGGSQVQLVESGGGLVKPGGSLRLSCAVSGFTFDDSDMGWYRQAPGNECELVSTITTDGSTYYADSVKGRFTISQDNAKTSAYLQMNSLRAEDTAVYYCAADLPILRPTPCGDSVLYNYWGQGTTVTVSS

SEQ ID NO: 73 - protein, 253 aa, homo sapiens
DIQMTQSPSSLSASVGDRVTITCRASQDIRNYLNWYQQKPGKAPKLLIYYTSRLESGVPSRFSGSGSGTDYTLTISSLQPEDFATYYCQQGNTLPWTFGQGTKVEIKGGGGSGGGGSGGGGSGGGGSGGGSEVQLVESGGGLVQPGGSLRLSCAASGYSFTGYTMNWVRQAPGKGLEWVALINPYKGVSTYNQKFKDRFTISVDKSKNTAYLQMNSLRAEDTAVYYCARSGYYGDSDWYFDVWGQGTLVTVSS

SEQ ID NO: 74 - protein, 498 aa, synthetic construct
EVQLVESGGGSVQTGETLRLSCTVSGFTFDDSDMGWYRQAPGNECELVSTITTDGSTYYADSVKGRFTISQDNAKTTAYLQMDSLKPEDTAVYYCAADLPILRPTPCGDSVLYNYWGQGTQVTVSSGGGGSGGGGSGGGGSEVQLVESGGGSVQTGETLRLSCTVSGFTFDDSDMGWYRQAPGNECELVSTITTDGSTYYADSVKGRFTISQDNAKTTAYLQMDSLKPEDTAVYYCAADLPILRPTPCGDSVLYNYWGQGTQVTVSSASERKSSVECPPCPAPEFEGGPSVFLFPPKPKDTLMISRTPEVTCVVVDVSQEDPEVQFNWYVDGVEVHNAKTKPREEQYNSTYRVVSVLTVLHQDWLNGKEYKCKVSNKALPASIEKTISKAKGQPREPQVCTLPPSQEEMTKNQVSLSCAVKGFYPSDIAVEWESNGQPENNYKTTPPVLDSDGSFFLVSKLTVDKSRWQEGNVFSCSVMHEALHNHYTQKSLSLSPGK

SEQ ID NO: 75 - protein, 741 aa, synthetic construct
DIQMTQSPSSLSASVGDRVTITCRASQDIRNYLNWYQQKPGKAPKLLIYYTSRLESGVPSRFSGSGSGTDYTLTISSLQPEDFATYYCQQGNTLPWTFGQGTKVEIKGGGGSGGGGSGGGGSGGGGSGGGSEVQLVESGGGLVQPGGSLRLSCAASGYSFTGYTMNWVRQAPGKGLEWVALINPYKGVSTYNQKFKDRFTISVDKSKNTAYLQMNSLRAEDTAVYYCARSGYYGDSDWYFDVWGQGTLVTVSSGGGGSDVKVTQSSRYLVKRTGEKVFLECVQDAPLSKMFWYRQDPGLGLRLIYFSYDVKMKEKGDIPEGYSVSREKKERFSLILESASTNQTSMYLCASSSDQNSGDPYEQYFGPGTRLTVTEDLKNVFPPEVAVFEPSKAEISRTQKATLVCLATGFYPPHVELSWWVNGKEVHDGVCTDPQPLKEQPALNDSRYALSSRLRVSATFWQDPRNHFRCQVQFYGLSENDEWTQDRAKPVTQIVSAEAWGRADCGGGGSASERKSCVECPPCPAPEFEGGPSVFLFPPKPKDTLMISRTPEVTCVVVDVSQEDPEVQFNWYVDGVEVHNAKTKPREEQYNSTYRVVSVLTVLHQDWLNGKEYKCKVSNKALPASIEKTISKAKGQPREPQVCTLPPSQEEMTKNQVSLSCAVKGFYPSDIAVEWESNGQPENNYKTTPPVLDSDGSFFLVSKLTVDKSRWQEGNVFSCSVMHEALHNHYTQKSLSLSPGK

SEQ ID NO: 76 - protein, 114 aa, synthetic construct
AQLVESGGGLVQPGGSLRLSCAASAYFSFKAMSWVRQAPGKGLEWVGSISPSGGSTYYNDNVLGRFTISRDNSKNTLYLQMNSLRAEDTAVYYCAKDVGFFDEWGQGTLVTVSS

SEQ ID NO: 77 - protein, 107 aa, synthetic construct
DIQMTQSPSSLSASVGDRVTITCRASQSISSYLAWYQQKPGKAPKLLIYDASIRDIGVPSRFSGSGSGTDFTLTISSLQPEDFATYYCQQYSSYPYTFGQGTKLEIK

SEQ ID NO: 78 - protein, 664 aa, synthetic construct
AQLVESGGGLVQPGGSLRLSCAASAYFSFKAMSWVRQAPGKGLEWVGSISPSGGSTYYNDNVLGRFTISRDNSKNTLYLQMNSLRAEDTAVYYCAKDVGFFDEWGQGTLVTVSSASTKGPSVFPLAPSSKSTSGGTAALGCLVEDYFPEPVTVSWNSGALTSGVHTFPAVLQSSGLYSLSSVVTVPSSSLGTQTYICNVNHKPSNTKVDEKVEPKSCDGGGGSGGGGSDIQMTQSPSSLSASVGDRVTITCRASQDIRNYLNWYQQKPGKAPKLLIYYTSRLESGVPSRFSGSGSGTDYTLTISSLQPEDFATYYCQQGNTLPWTFGQGTKVEIKSSASTKGPSVFPLAPSSKSTSGGTAALGCLVKDYFPEPVTVSWNSGALTSGVHTFPAVLQSSGLYSLSSVVTVPSSSLGTQTYICNVNHKPSNTKVDKRVERKSCVECPPCPAPEFEGGPSVFLFPPKPKDTLMISRTPEVTCVVVDVSHEDPEVKFNWYVDGVEVHNAKTKPREEQYNSTYRVVSVLTVLHQDWLNGKEYKCKVSNKALPASIEKTISKAKGQPREPQVYTLPPCREEMTKNQVSLWCLVKGFYPSDIAVEWESNGQPENNYKTTPPVLDSDGSFFLYSKLTVDKSRWQQGNVFSCSVMHEALHNHYTQKSLSLSPGK

SEQ ID NO: 79 - protein, 441 aa, synthetic construct
AQLVESGGGLVQPGGSLRLSCAASAYFSFKAMSWVRQAPGKGLEWVGSISPSGGSTYYNDNVLGRFTISRDNSKNTLYLQMNSLRAEDTAVYYCAKDVGFFDEWGQGTLVTVSSASTKGPSVFPLAPSSKSTSGGTAALGCLVEDYFPEPVTVSWNSGALTSGVHTFPAVLQSSGLYSLSSVVTVPSSSLGTQTYICNVNHKPSNTKVDEKVERKSCVECPPCPAPEFEGGPSVFLFPPKPKDTLMISRTPEVTCVVVDVSQEDPEVQFNWYVDGVEVHNAKTKPREEQYNSTYRVVSVLTVLHQDWLNGKEYKCKVSNKALPASIEKTISKAKGQPREPQVCTLPPSQEEMTKNQVSLSCAVKGFYPSDIAVEWESNGQPENNYKTTPPVLDSDGSFFLVSKLTVDKSRWQEGNVFSCSVMHEALHNHYTQKSLSLSPGK

SEQ ID NO: 80 - protein, 214 aa, synthetic construct
DIQMTQSPSSLSASVGDRVTITCRASQSISSYLAWYQQKPGKAPKLLIYDASIRDIGVPSRFSGSGSGTDFTLTISSLQPEDFATYYCQQYSSYPYTFGQGTKLEIKRTVAAPSVFIFPPSDRKLKSGTASVVCLLNNFYPREAKVQWKVDNALQSGNSQESVTEQDSKDSTYSLSSTLTLSKADYEKHKVYACEVTHQGLSSPVTKSFNRGEC

SEQ ID NO: 81 - protein, 229 aa, synthetic construct
EVQLVESGGGLVQPGGSLRLSCAASGYSFTGYTMNWVRQAPGKGLEWVALINPYKGVSTYNQKFKDRFTISVDKSKNTAYLQMNSLRAEDTAVYYCARSGYYGDSDWYFDVWGQGTLVTVSSASVAAPSVFIFPPSDEQLKSGTASVVCLLNNFYPREAKVQWKVDNALQSGNSQESVTEQDSKDSTYSLSSTLTLSKADYEKHKVYACEVTHQGLSSPVTKSFNRGEC

SEQ ID NO: 82 - protein, 10 aa, synthetic construct
AVYDGREHTV

SEQ ID NO: 83 - protein, 10 aa, synthetic construct
GAYDGREHTV

SEQ ID NO: 84 - protein, 10 aa, synthetic construct
GVADGREHTV

SEQ ID NO: 85 - protein, 10 aa, synthetic construct
GVYAGREHTV

SEQ ID NO: 86 - protein, 10 aa, synthetic construct
GVYDAREHTV

SEQ ID NO: 87 - protein, 10 aa, synthetic construct
GVYDGAEHTV

SEQ ID NO: 88 - protein, 10 aa, synthetic construct
GVYDGRAHTV

SEQ ID NO: 89 - protein, 10 aa, synthetic construct
GVYDGREATV

SEQ ID NO: 90 - protein, 10 aa, synthetic construct
GVYDGREHAV

SEQ ID NO: 91 - protein, 10 aa, synthetic construct
GVYDGREHTA

SEQ ID NO: 92 - protein, 231 aa, synthetic construct
ASERKSSVECPPCPAPEFEGGPSVFLFPPKPKDTLMISRTPEVTCVVVDVSQEDPEVQFNWYVDGVEVHNAKTKPREEQYNSTYRVVSVLTVLHQDWLNGKEYKCKVSNKALPASIEKTISKAKGQPREPQVCTLPPSQEEMTKNQVSLSCAVKGFYPSDIAVEWESNGQPENNYKTTPPVLDSDGSFFLVSKLTVDKSRWQEGNVFSCSVMHEALHNHYTQKSLSLSPGK

SEQ ID NO: 93 - protein, 231 aa, synthetic construct
ASERKSSVECPPCPAPEFEGGPSVFLFPPKPKDTLMISRTPEVTCVVVDVSHEDPEVKFNWYVDGVEVHNAKTKPREEQYNSTYRVVSVLTVLHQDWLNGKEYKCKVSNKALPASIEKTISKAKGQPREPQVYTLPPCREEMTKNQVSLWCLVKGFYPSDIAVEWESNGQPENNYKTTPPVLDSDGSFFLYSKLTVDKSRWQQGNVFSCSVMHEALHNHYTQKSLSLSPGK

SEQ ID NO: 94 - protein, 318 aa, Homo sapiens
MLLGQKSQRYKAEEGLQAQGEAPGLMDVQIPTAEEQKAASSSSTLIMGTLEEVTDSGSPSPPQSPEGASSSLTVTDSTLWSQSDEGSSSNEEEGPSTSPDPAHLESLFREALDEKVAELVRFLLRKYQIKEPVTKAEMLESVIKNYKNHFPDIFSKASECMQVIFGIDVKEVDPAGHSYILVTCLGLSYDGLLGDDQSTPKTGLLIIVLGMILMEGSRAPEEAIWEALSVMGLYDGREHSVYWKLRKLLTQEWVQENYLEYRQAPGSDPVRYEFLWGPRALAETSYVKVLEHVVRVNARVRISYPSLHEEALGEEKGV